European Patent Application EP 4 674 424 A1, published January 7, 2026. Title: Anti-Aging Composition Comprising Peptide Complex As Active Ingredient. Applicant: CAREGEN CO., LTD. The sequence listing filed with the application follows.

SEQUENCE LISTING (12 sequences)

SEQ ID NO: 1 - protein, 5 aa, synthetic construct
LKTRN

SEQ ID NO: 2 - protein, 9 aa, synthetic construct
KGSATGWMA

SEQ ID NO: 3 - DNA, 20 bp, synthetic construct
  source 1..20: mol_type = other DNA
cgtctgcctcagaaggactc

SEQ ID NO: 4 - DNA, 20 bp, synthetic construct
  source 1..20: mol_type = other DNA
tctaccatgctcagggggtc

SEQ ID NO: 5 - DNA, 20 bp, synthetic construct
  source 1..20: mol_type = other DNA
gatcctttggattcctgcaa

SEQ ID NO: 6 - DNA, 20 bp, synthetic construct
  source 1..20: mol_type = other DNA
agttccagccgtctctgtgt

SEQ ID NO: 7 - DNA, 20 bp, synthetic construct
  source 1..20: mol_type = other DNA
tcaccggacataaagtggct

SEQ ID NO: 8 - DNA, 20 bp, synthetic construct
  source 1..20: mol_type = other DNA
tgatgatgtgagggtgcctg

SEQ ID NO: 9 - DNA, 24 bp, synthetic construct
  source 1..24: mol_type = other DNA
ccccatcggggttgatgatccacc

SEQ ID NO: 10 - DNA, 21 bp, synthetic construct
  source 1..21: mol_type = other DNA
tttgtcccagatctacgagtg

SEQ ID NO: 11 - DNA, 20 bp, synthetic construct
  source 1..20: mol_type = other DNA
gtgatggcatggactgtggt

SEQ ID NO: 12 - DNA, 20 bp, synthetic construct
  source 1..20: mol_type = other DNA
ggagccaaaagggtcatcat